European Patent Specification EP 3 883 966 B1, published July 12, 2023. Title: HUMANIZED ANTI-HUMAN-PD-1 ANTIBODY. Applicant: OSE IMMUNOTHERAPEUTICS. The sequence listing filed with the application follows.

SEQUENCE LISTING (51 sequences)

SEQ ID NO: 1 - protein, 5 aa, artificial
  HC CDR1
HYAMN

SEQ ID NO: 2 - protein, 17 aa, artificial
  HC CDR2
WINTNTGEPTYAQGFTG

SEQ ID NO: 3 - protein, 8 aa, artificial
  HC CDR3
EREPGMDS

SEQ ID NO: 4 - protein, 8 aa, artificial
  HC CDR3
EREPGMDT

SEQ ID NO: 5 - protein, 8 aa, artificial
  HC CDR3
EREPGMES

SEQ ID NO: 6 - protein, 8 aa, artificial
  HC CDR3
EREPGMDH

SEQ ID NO: 7 - protein, 8 aa, artificial
  HC CDR3
EREPGMDA

SEQ ID NO: 8 - protein, 8 aa, artificial
  HC CDR3
EREPGMDY

SEQ ID NO: 9 - protein, 8 aa, artificial
  HC CDR3
EREPGMDN

SEQ ID NO: 10 - protein, 8 aa, artificial
  HC CDR3
EREPGMDE

SEQ ID NO: 11 - protein, 16 aa, artificial
  LC CDR1
RSSQSLVHANGNTYLE

SEQ ID NO: 12 - protein, 16 aa, artificial
  LC CDR1
RSSQSLVHANTNTYLE

SEQ ID NO: 13 - protein, 7 aa, artificial
  LC CDR2
KVSNRFS

SEQ ID NO: 14 - protein, 9 aa, artificial
  LC CDR3
FQGTHVPNT

SEQ ID NO: 15 - protein, 117 aa, artificial
  HC variable domain
QIQLVQSGSELKKPGASVKVSCKASGYTFTHYAMNWVRQAPGQGLEWMGWINTNTGEPTYAQGFTGRFVFSLDTSVSTAYLQISSLKAEDTAVYYCAREREPGMDSWGQGTLVTVSS

SEQ ID NO: 16 - protein, 117 aa, artificial
  HC variable domain
QIQLVQSGSELKKPGASVKVSCKASGYTFTHYAMNWVRQAPGQGLEWMGWINTNTGEPTYAQGFTGRFVFSLDTSVSTAYLQISSLKAEDTAVYYCAREREPGMDTWGQGTLVTVSS

SEQ ID NO: 17 - protein, 117 aa, artificial
  HC variable domain
QIQLVQSGSELKKPGASVKVSCKASGYTFTHYAMNWVRQAPGQGLEWMGWINTNTGEPTYAQGFTGRFVFSLDTSVSTAYLQISSLKAEDTAVYYCAREREPGMESWGQGTLVTVSS

SEQ ID NO: 18 - protein, 117 aa, artificial
  HC variable domain
QIQLVQSGSELKKPGASVKVSCKASGYTFTHYAMNWVRQAPGQGLEWMGWINTNTGEPTYAQGFTGRFVFSLDTSVSTAYLQISSLKAEDTAVYYCAREREPGMDHWGQGTLVTVSS

SEQ ID NO: 19 - protein, 117 aa, artificial
  HC variable domain
QIQLVQSGSELKKPGASVKVSCKASGYTFTHYAMNWVRQAPGQGLEWMGWINTNTGEPTYAQGFTGRFVFSLDTSVSTAYLQISSLKAEDTAVYYCAREREPGMDAWGQGTLVTVSS

SEQ ID NO: 20 - protein, 117 aa, artificial
  HC variable domain
QIQLVQSGSELKKPGASVKVSCKASGYTFTHYAMNWVRQAPGQGLEWMGWINTNTGEPTYAQGFTGRFVFSLDTSVSTAYLQISSLKAEDTAVYYCAREREPGMDYWGQGTLVTVSS

SEQ ID NO: 21 - protein, 117 aa, artificial
  HC variable domain
QIQLVQSGSELKKPGASVKVSCKASGYTFTHYAMNWVRQAPGQGLEWMGWINTNTGEPTYAQGFTGRFVFSLDTSVSTAYLQISSLKAEDTAVYYCAREREPGMDNWGQGTLVTVSS

SEQ ID NO: 22 - protein, 117 aa, artificial
  HC variable domain
QIQLVQSGSELKKPGASVKVSCKASGYTFTHYAMNWVRQAPGQGLEWMGWINTNTGEPTYAQGFTGRFVFSLDTSVSTAYLQISSLKAEDTAVYYCAREREPGMDEWGQGTLVTVSS

SEQ ID NO: 23 - protein, 112 aa, artificial
  LC variable domain
DVVMTQSPLSLPVTLGQPASISCRSSQSLVHANGNTYLEWYQQRPGQSPRLLIYKVSNRFSGVPDRFSGSGSGTDFTLKISRVEAEDVGVYYCFQGTHVPNTFGQGTKLEIK

SEQ ID NO: 24 - protein, 112 aa, artificial
  LC variable domain
DVVMTQSPLSLPVTLGQPASISCRSSQSLVHANTNTYLEWYQQRPGQSPRLLIYKVSNRFSGVPDRFSGSGSGTDFTLKISRVEAEDVGVYYCFQGTHVPNTFGQGTKLEIK

SEQ ID NO: 25 - protein, 444 aa, artificial
  HC
QIQLVQSGSELKKPGASVKVSCKASGYTFTHYAMNWVRQAPGQGLEWMGWINTNTGEPTYAQGFTGRFVFSLDTSVSTAYLQISSLKAEDTAVYYCAREREPGMDSWGQGTLVTVSSASTKGPSVFPLAPCSRSTSESTAALGCLVKDYFPEPVTVSWNSGALTSGVHTFPAVLQSSGLYSLSSVVTVPSSSLGTKTYTCNVDHKPSNTKVDKRVESKYGPPCPPCPAPEFLGGPSVFLFPPKPKDTLMISRTPEVTCVVVDVSQEDPEVQFNWYVDGVEVHNAKTKPREEQFNSTYRVVSVLTVLHQDWLNGKEYKCKVSNKGLPSSIEKTISKAKGQPREPQVYTLPPSQEEMTKNQVSLTCLVKGFYPSDIAVEWESNGQPENNYKTTPPVLDSDGSFFLYSRLTVDKSRWQEGNVFSCSVMHEALHNHYTQKSLSLSPGK

SEQ ID NO: 26 - protein, 444 aa, artificial
  HC
QIQLVQSGSELKKPGASVKVSCKASGYTFTHYAMNWVRQAPGQGLEWMGWINTNTGEPTYAQGFTGRFVFSLDTSVSTAYLQISSLKAEDTAVYYCAREREPGMDTWGQGTLVTVSSASTKGPSVFPLAPCSRSTSESTAALGCLVKDYFPEPVTVSWNSGALTSGVHTFPAVLQSSGLYSLSSVVTVPSSSLGTKTYTCNVDHKPSNTKVDKRVESKYGPPCPPCPAPEFLGGPSVFLFPPKPKDTLMISRTPEVTCVVVDVSQEDPEVQFNWYVDGVEVHNAKTKPREEQFNSTYRVVSVLTVLHQDWLNGKEYKCKVSNKGLPSSIEKTISKAKGQPREPQVYTLPPSQEEMTKNQVSLTCLVKGFYPSDIAVEWESNGQPENNYKTTPPVLDSDGSFFLYSRLTVDKSRWQEGNVFSCSVMHEALHNHYTQKSLSLSPGK

SEQ ID NO: 27 - protein, 444 aa, artificial
  HC
QIQLVQSGSELKKPGASVKVSCKASGYTFTHYAMNWVRQAPGQGLEWMGWINTNTGEPTYAQGFTGRFVFSLDTSVSTAYLQISSLKAEDTAVYYCAREREPGMESWGQGTLVTVSSASTKGPSVFPLAPCSRSTSESTAALGCLVKDYFPEPVTVSWNSGALTSGVHTFPAVLQSSGLYSLSSVVTVPSSSLGTKTYTCNVDHKPSNTKVDKRVESKYGPPCPPCPAPEFLGGPSVFLFPPKPKDTLMISRTPEVTCVVVDVSQEDPEVQFNWYVDGVEVHNAKTKPREEQFNSTYRVVSVLTVLHQDWLNGKEYKCKVSNKGLPSSIEKTISKAKGQPREPQVYTLPPSQEEMTKNQVSLTCLVKGFYPSDIAVEWESNGQPENNYKTTPPVLDSDGSFFLYSRLTVDKSRWQEGNVFSCSVMHEALHNHYTQKSLSLSPGK

SEQ ID NO: 28 - protein, 444 aa, artificial
  HC
QIQLVQSGSELKKPGASVKVSCKASGYTFTHYAMNWVRQAPGQGLEWMGWINTNTGEPTYAQGFTGRFVFSLDTSVSTAYLQISSLKAEDTAVYYCAREREPGMDHWGQGTLVTVSSASTKGPSVFPLAPCSRSTSESTAALGCLVKDYFPEPVTVSWNSGALTSGVHTFPAVLQSSGLYSLSSVVTVPSSSLGTKTYTCNVDHKPSNTKVDKRVESKYGPPCPPCPAPEFLGGPSVFLFPPKPKDTLMISRTPEVTCVVVDVSQEDPEVQFNWYVDGVEVHNAKTKPREEQFNSTYRVVSVLTVLHQDWLNGKEYKCKVSNKGLPSSIEKTISKAKGQPREPQVYTLPPSQEEMTKNQVSLTCLVKGFYPSDIAVEWESNGQPENNYKTTPPVLDSDGSFFLYSRLTVDKSRWQEGNVFSCSVMHEALHNHYTQKSLSLSPGK

SEQ ID NO: 29 - protein, 444 aa, artificial
  HC
QIQLVQSGSELKKPGASVKVSCKASGYTFTHYAMNWVRQAPGQGLEWMGWINTNTGEPTYAQGFTGRFVFSLDTSVSTAYLQISSLKAEDTAVYYCAREREPGMDAWGQGTLVTVSSASTKGPSVFPLAPCSRSTSESTAALGCLVKDYFPEPVTVSWNSGALTSGVHTFPAVLQSSGLYSLSSVVTVPSSSLGTKTYTCNVDHKPSNTKVDKRVESKYGPPCPPCPAPEFLGGPSVFLFPPKPKDTLMISRTPEVTCVVVDVSQEDPEVQFNWYVDGVEVHNAKTKPREEQFNSTYRVVSVLTVLHQDWLNGKEYKCKVSNKGLPSSIEKTISKAKGQPREPQVYTLPPSQEEMTKNQVSLTCLVKGFYPSDIAVEWESNGQPENNYKTTPPVLDSDGSFFLYSRLTVDKSRWQEGNVFSCSVMHEALHNHYTQKSLSLSPGK

SEQ ID NO: 30 - protein, 444 aa, artificial
  HC
QIQLVQSGSELKKPGASVKVSCKASGYTFTHYAMNWVRQAPGQGLEWMGWINTNTGEPTYAQGFTGRFVFSLDTSVSTAYLQISSLKAEDTAVYYCAREREPGMDYWGQGTLVTVSSASTKGPSVFPLAPCSRSTSESTAALGCLVKDYFPEPVTVSWNSGALTSGVHTFPAVLQSSGLYSLSSVVTVPSSSLGTKTYTCNVDHKPSNTKVDKRVESKYGPPCPPCPAPEFLGGPSVFLFPPKPKDTLMISRTPEVTCVVVDVSQEDPEVQFNWYVDGVEVHNAKTKPREEQFNSTYRVVSVLTVLHQDWLNGKEYKCKVSNKGLPSSIEKTISKAKGQPREPQVYTLPPSQEEMTKNQVSLTCLVKGFYPSDIAVEWESNGQPENNYKTTPPVLDSDGSFFLYSRLTVDKSRWQEGNVFSCSVMHEALHNHYTQKSLSLSPGK

SEQ ID NO: 31 - protein, 444 aa, artificial
  HC
QIQLVQSGSELKKPGASVKVSCKASGYTFTHYAMNWVRQAPGQGLEWMGWINTNTGEPTYAQGFTGRFVFSLDTSVSTAYLQISSLKAEDTAVYYCAREREPGMDNWGQGTLVTVSSASTKGPSVFPLAPCSRSTSESTAALGCLVKDYFPEPVTVSWNSGALTSGVHTFPAVLQSSGLYSLSSVVTVPSSSLGTKTYTCNVDHKPSNTKVDKRVESKYGPPCPPCPAPEFLGGPSVFLFPPKPKDTLMISRTPEVTCVVVDVSQEDPEVQFNWYVDGVEVHNAKTKPREEQFNSTYRVVSVLTVLHQDWLNGKEYKCKVSNKGLPSSIEKTISKAKGQPREPQVYTLPPSQEEMTKNQVSLTCLVKGFYPSDIAVEWESNGQPENNYKTTPPVLDSDGSFFLYSRLTVDKSRWQEGNVFSCSVMHEALHNHYTQKSLSLSPGK

SEQ ID NO: 32 - protein, 444 aa, artificial
  HC
QIQLVQSGSELKKPGASVKVSCKASGYTFTHYAMNWVRQAPGQGLEWMGWINTNTGEPTYAQGFTGRFVFSLDTSVSTAYLQISSLKAEDTAVYYCAREREPGMDEWGQGTLVTVSSASTKGPSVFPLAPCSRSTSESTAALGCLVKDYFPEPVTVSWNSGALTSGVHTFPAVLQSSGLYSLSSVVTVPSSSLGTKTYTCNVDHKPSNTKVDKRVESKYGPPCPPCPAPEFLGGPSVFLFPPKPKDTLMISRTPEVTCVVVDVSQEDPEVQFNWYVDGVEVHNAKTKPREEQFNSTYRVVSVLTVLHQDWLNGKEYKCKVSNKGLPSSIEKTISKAKGQPREPQVYTLPPSQEEMTKNQVSLTCLVKGFYPSDIAVEWESNGQPENNYKTTPPVLDSDGSFFLYSRLTVDKSRWQEGNVFSCSVMHEALHNHYTQKSLSLSPGK

SEQ ID NO: 33 - protein, 219 aa, artificial
  LC
DVVMTQSPLSLPVTLGQPASISCRSSQSLVHANGNTYLEWYQQRPGQSPRLLIYKVSNRFSGVPDRFSGSGSGTDFTLKISRVEAEDVGVYYCFQGTHVPNTFGQGTKLEIKRTVAAPSVFIFPPSDEQLKSGTASVVCLLNNFYPREAKVQWKVDNALQSGNSQESVTEQDSKDSTYSLSSTLTLSKADYEKHKVYACEVTHQGLSSPVTKSFNRGEC

SEQ ID NO: 34 - protein, 219 aa, artificial
  LC
DVVMTQSPLSLPVTLGQPASISCRSSQSLVHANTNTYLEWYQQRPGQSPRLLIYKVSNRFSGVPDRFSGSGSGTDFTLKISRVEAEDVGVYYCFQGTHVPNTFGQGTKLEIKRTVAAPSVFIFPPSDEQLKSGTASVVCLLNNFYPREAKVQWKVDNALQSGNSQESVTEQDSKDSTYSLSSTLTLSKADYEKHKVYACEVTHQGLSSPVTKSFNRGEC

SEQ ID NO: 35 - protein, 327 aa, artificial
  HC constant domain
ASTKGPSVFPLAPCSRSTSESTAALGCLVKDYFPEPVTVSWNSGALTSGVHTFPAVLQSSGLYSLSSVVTVPSSSLGTKTYTCNVDHKPSNTKVDKRVESKYGPPCPPCPAPEFLGGPSVFLFPPKPKDTLMISRTPEVTCVVVDVSQEDPEVQFNWYVDGVEVHNAKTKPREEQFNSTYRVVSVLTVLHQDWLNGKEYKCKVSNKGLPSSIEKTISKAKGQPREPQVYTLPPSQEEMTKNQVSLTCLVKGFYPSDIAVEWESNGQPENNYKTTPPVLDSDGSFFLYSRLTVDKSRWQEGNVFSCSVMHEALHNHYTQKSLSLSPGK

SEQ ID NO: 36 - protein, 107 aa, artificial [sequence omitted]

SEQ ID NO: 37 - protein, 30 aa, artificial
  HFR1
QIQLVQSGSELKKPGASVKVSCKASGYTFT

SEQ ID NO: 38 - protein, 14 aa, artificial
  HFR2
WVRQAPGQGLEWMG

SEQ ID NO: 39 - protein, 32 aa, artificial
  HFR3
RFVFSLDTSVSTAYLQISSLKAEDTAVYYCAR

SEQ ID NO: 40 - protein, 11 aa, artificial
  HFR4
WGQGTLVTVSS

SEQ ID NO: 41 - protein, 23 aa, artificial
  LFR1
DVVMTQSPLSLPVTLGQPASISC

SEQ ID NO: 42 - protein, 15 aa, artificial
  LFR2
WYQQRPGQSPRLLIY

SEQ ID NO: 43 - protein, 32 aa, artificial
  LFR3
GVPDRFSGSGSGTDFTLKISRVEAEDVGVYYC

SEQ ID NO: 44 - protein, 10 aa, artificial
  LFR4
FGQGTKLEIK

SEQ ID NO: 45 - protein, 19 aa, artificial
  signal peptide
MDWLWNLLFLMAAAQSIQA

SEQ ID NO: 46 - protein, 19 aa, artificial
  signal peptide
MKLPVRLLVLMFWIPASSS

SEQ ID NO: 47 - protein, 330 aa, artificial
  IgG1m-N298A
ASTKGPSVFPLAPSSKSTSGGTAALGCLVKDYFPEPVTVSWNSGALTSGVHTFPAVLQSSGLYSLSSVVTVPSSSLGTQTYICNVNHKPSNTKVDKKVEPKSCDKTHTCPPCPAPELLGGPSVFLFPPKPKDTLMISRTPEVTCVVVDVSHEDPEVKFNWYVDGVEVHNAKTKPREEQYASTYRVVSVLTVLHQDWLNGKEYKCKVSNKALPAPIEKTISKAKGQPREPQVYTLPPSRDELTKNQVSLTCLVKGFYPSDIAVEWESNGQPENNYKTTPPVLDSDGSFFLYSKLTVDKSRWQQGNVFSCSVMHEALHNHYTQKSLSLSPGK

SEQ ID NO: 48 - DNA, 351 bp, artificial
  VH HK
cagatccagctggtgcagagcggctctgagctgaagaagccaggcgcttctgtgaaggtgtcctgcaaggccagcggctacaccttcacacactatgctatgaattgggtgagacaggctccaggacagggactggagtggatgggctggatcaacaccaatacaggcgagcctacctacgctcagggctttacaggccgcttcgtgttttctctggatacctccgtgagcacagcctatctgcagatctccagcctgaaggctgaggacaccgccgtgtactattgtgctagggagagggagccaggaatggataactggggacagggcaccctggtgacagtgtcttcc

SEQ ID NO: 49 - DNA, 336 bp, artificial
  VL LD
gacgtggtcatgacacagagcccactgtctctgcctgtgaccctgggacagccagcctctatctcctgcagatccagccagtctctggtgcacgctaacaccaatacatacctggagtggtatcagcagaggccaggacagtccccaaggctgctgatctacaaggtgtccaacagattcagcggagtgccagaccgctttagcggatctggatccggaaccgacttcaccctgaagatctccagggtggaggctgaggatgtgggcgtgtactattgtttccagggcacccatgtgcctaatacatttggccagggcaccaagctggagatcaag

SEQ ID NO: 50 - DNA, 1335 bp, artificial
  CH HK
cagatccagctggtgcagagcggctctgagctgaagaagccaggcgcttctgtgaaggtgtcctgcaaggccagcggctacaccttcacacactatgctatgaattgggtgagacaggctccaggacagggactggagtggatgggctggatcaacaccaatacaggcgagcctacctacgctcagggctttacaggccgcttcgtgttttctctggatacctccgtgagcacagcctatctgcagatctccagcctgaaggctgaggacaccgccgtgtactattgtgctagggagagggagccaggaatggataactggggacagggcaccctggtgacagtgtcttccgctagcaccaagggcccatcggtcttccccctggcgccctgctccaggagcacctccgagagcacagccgccctgggctgcctggtcaaggactacttccccgaaccggtgacggtgtcgtggaactcaggcgccctgaccagcggcgtgcacaccttcccggctgtcctacagtcctcaggactctactccctcagcagcgtggtgaccgtgccctccagcagcttgggcacgaagacctacacctgcaacgtagatcacaagcccagcaacaccaaggtggacaagagagttgagtccaaatatggtcccccatgcccaccatgcccagcacctgagttcctggggggaccatcagtcttcctgttccccccaaaacccaaggacactctcatgatctcccggacccctgaggtcacgtgcgtggtggtggacgtgagccaggaagaccccgaggtccagttcaactggtacgtggatggcgtggaggtgcataatgccaagacaaagccgcgggaggagcagttcaacagcacgtaccgtgtggtcagcgtcctcaccgtcctgcaccaggactggctgaacggcaaggagtacaagtgcaaggtctccaacaaaggcctcccgtcctccatcgagaaaaccatctccaaagccaaagggcagccccgagagccacaggtgtacaccctgcccccatcccaggaggagatgaccaagaaccaggtcagcctgacctgcctggtcaaaggcttctaccccagcgacatcgccgtggagtgggagagcaatgggcagccggagaacaactacaagaccacgcctcccgtgctggactccgacggctccttcttcctctacagcaggctaaccgtggacaagagcaggtggcaggaggggaatgtcttctcatgctccgtgatgcatgaggctctgcacaaccactacacacagaagagcctctccctgtctccgggtaaatga

SEQ ID NO: 51 - DNA, 660 bp, artificial
  CL LD
gacgtggtcatgacacagagcccactgtctctgcctgtgaccctgggacagccagcctctatctcctgcagatccagccagtctctggtgcacgctaacaccaatacatacctggagtggtatcagcagaggccaggacagtccccaaggctgctgatctacaaggtgtccaacagattcagcggagtgccagaccgctttagcggatctggatccggaaccgacttcaccctgaagatctccagggtggaggctgaggatgtgggcgtgtactattgtttccagggcacccatgtgcctaatacatttggccagggcaccaagctggagatcaagcgtacggtggctgcaccatctgtcttcatcttcccgccatctgatgagcagttgaaatctggaactgcctctgttgtgtgcctgctgaataacttctatcccagagaggccaaagtacagtggaaggtggataacgccctccaatcgggtaactcccaggagagtgtcacagagcaggacagcaaggacagcacctacagcctcagcagcaccctgacgctgagcaaagcagactacgagaaacacaaagtctacgcctgcgaagtcacccatcagggcctgagctcgcccgtcacaaagagcttcaacaggggagagtgttag